European Patent Application EP 4 800 123 A1, published September 2, 2026. Title: Internal control nucleic acid, method for designing said nucleic acid, and kit comprising said nucleic acid. Applicant: Kanto Kagaku Kabushiki Kaisha. Application EP. The sequence listing filed with the application follows.

SEQUENCE LISTING (14 sequences)

SEQ ID NO: 1 - DNA, 1000 bp, synthetic construct
  source 1..1000: mol_type = other DNA
gcacatgtgctgacccagattagacgtgagatgaaggtcttgtaaaccaggtcaagtactcttgaagtgacacgatccacgatgtccaccgttgggacgtgagttccaacggtgtaaggtgaagatccgtgacttctcatggaagcacgatggacttgcacatatctattctgacacggagtctagaggagctagtctcttaggtgcgaccaggattagtcccaacattacgggagtcgtcaattagacgtctatccatggcagaatcctaatgggtaccgagatggagtcgaacctctctagtcctaagctcgagagcgatggttctatcggattctgctacctatgatcgtaaggacttaatacgctggggtcaactagtaatgtgccagtggcatagtttcatgcagatactgctccgctaagtggctcaagggtcagttgatatcttgcaccgttcagccatctccctagcatgcacacaaagttctcttatgtacggacttcgccacgaactaacaatctggtgtagcatcatccactgacgcgaatgcattccgctatcatcaccatatagtggtgcttgtatgaggtcaagtccctgattaatccgcataagcaatcctttgggctacacccagttagattagcgatcagggatgtattcattcatgagtaggctagtggctggaacttctatgcccatctacgtcctctacaagacagctcgtcataagttgagtatacggaccggaccaagattggattgctcactggtcgcgatgtgcaatctctaccgagtttctcgtaccgaaggtacgatcttcccatagacgcatacatcgaggatcgaactgccttaaatgacggaacgccattactaggctcatcgacgcgctacggtatgttcaactcaggagaccttctctacccatcgttaacgtgctgaactaatcaggttcgacaatctcgattgatacacggatcggaattggcttag

SEQ ID NO: 2 - DNA, 19 bp, synthetic construct
  source 1..19: mol_type = other DNA
taagtggctcaagggtcag

SEQ ID NO: 3 - DNA, 20 bp, synthetic construct
  source 1..20: mol_type = other DNA
cctagcatgcacacaaagtt

SEQ ID NO: 4 - DNA, 24 bp, synthetic construct
  source 1..24: mol_type = other DNA
tatcttgcaccgttcagccatctc

SEQ ID NO: 5 - DNA, 16 bp, synthetic construct
  source 1..16: mol_type = other DNA
gcttcggtccagtaga

SEQ ID NO: 6 - DNA, 20 bp, synthetic construct
  source 1..20: mol_type = other DNA
gttgtgtacgtcccgtctgc

SEQ ID NO: 7 - DNA, 24 bp, synthetic construct
  source 1..24: mol_type = other DNA
ttctatcctggtgctgcgcattcg

SEQ ID NO: 8 - DNA, 20 bp, synthetic construct
  source 1..20: mol_type = other DNA
gtgagctccactgtgacaag

SEQ ID NO: 9 - DNA, 20 bp, synthetic construct
  source 1..20: mol_type = other DNA
cacacaccatcatcgaaact

SEQ ID NO: 10 - DNA, 22 bp, synthetic construct
  source 1..22: mol_type = other DNA
cttcccctggctattctgctca

SEQ ID NO: 11 - DNA, 124 bp, synthetic construct
  source 1..124: mol_type = other DNA
taatacgactcactatagagggtcatcgtctttttctaggacattgtattgaacagcagctgtgtatgtggagccttcgtgaagcttgttcacgtatgtttccatatttgccccacccctcgag

SEQ ID NO: 12 - DNA, 24 bp, synthetic construct
  source 1..24: mol_type = other DNA
ggcaaatatggaaacatacgtgaa

SEQ ID NO: 13 - DNA, 28 bp, synthetic construct
  source 1..28: mol_type = other DNA
tctttttctaggacattgtaytgaacag

SEQ ID NO: 14 - DNA, 28 bp, synthetic construct
  source 1..28: mol_type = other DNA
tctttttctaggacattgtaytgaacag